European Patent Application EP 4 365 191 A1, published May 8, 2024. Title: Recombinant botulinum toxin type A light chain, recombinant botulinum toxin, and its compositions, uses and methods. Applicant: Medytox Inc. The sequence listing filed with the application follows.

SEQUENCE LISTING (41 sequences)

SEQ ID NO: 1 - protein, 120 aa, Clostridium botulinum
MPFVNKQFNYKDPVNGVDIAYIKIPNAGQMQPVKAFKIHNKIWVIPERDTFTNPEEGDLNPPPEAKQVPVSYYDSTYLSTDNEKDNYLKGVTKLFERIYSTDLGRMLLTSIVRGIPFWGG

SEQ ID NO: 2 - protein, 120 aa, Clostridium botulinum
STIDTELKVIDTNCINVIQPDGSYRSEELNLVIIGPSADIIQFECKSFGHEVLNLTRNGYGSTQYIRFSPDFTFGFEESLEVDTNPLLGAGKFATDPAVTLAHELIHAGHRLYGIAINPN

SEQ ID NO: 3 - protein, 156 aa, Clostridium botulinum
RVFKVNTNAYYEMSGLEVSFEELRTFGGHDAKFIDSLQENEFRLYYYNKFKDIASTLNKAKSIVGTTASLQYMKNVFKEKYLLSEDTSGKFSVDKLKFDKLYKMLTEIYTEDNFVKFFKVLNRKTYLNFDKAVFKINIVPKVNYTIYDGFNLRNTN

SEQ ID NO: 4 - protein, 29 aa, Clostridium botulinum
LAANFNGQNTEINNMNFTKLKNFTGLFEF

SEQ ID NO: 5 - protein, 120 aa, Clostridium botulinum
MPFVNKQFNYNDPENGVDIAYIKIPNAGKMQPVKAFKIHNKVWVIPERDIFTNPEEVDLNPPPEAKQVPISYYDSAYLSTDNEKDNYLKGVIKLFERIYSTDLGRMLLISIVRGIPFWGG

SEQ ID NO: 6 - protein, 120 aa, Clostridium botulinum
GKIDTELKVIDTNCINIIQLDDSYRSEELNLAIIGPSANIIESQCSSFRDDVLNLTRNGYGSTQYIRFSPDFTVGFEESLEVDTNPLLGAGKFAQDPAVALAHELIHAEHRLYGIAINTN

SEQ ID NO: 7 - protein, 156 aa, Clostridium botulinum
RVFKVNTNAYYEMAGLEVSLEELITFGGNDAKFIDSLQKKEFSLYYYNKFKDIASTLNKAKSIVGTTASLQYMKNVFKEKYLLSEDATGKFLVDRLKFDELYKLLTEIYTEDNFVKFFKVLNRKTYLNFDKAVFKINIVPDVNYTIHDGFNLRNTN

SEQ ID NO: 8 - protein, 29 aa, Clostridium botulinum
LAANFNGQNIEINNKNFDKLKNFTGLFEF

SEQ ID NO: 9 - protein, 425 aa, Clostridium botulinum
MPFVNKQFNYKDPVNGVDIAYIKIPNAGQMQPVKAFKIHNKIWVIPERDTFTNPEEGDLNPPPEAKQVPVSYYDSTYLSTDNEKDNYLKGVTKLFERIYSTDLGRMLLTSIVRGIPFWGGSTIDTELKVIDTNCINVIQPDGSYRSEELNLVIIGPSADIIQFECKSFGHEVLNLTRNGYGSTQYIRFSPDFTFGFEESLEVDTNPLLGAGKFATDPAVTLAHELIHAGHRLYGIAINPNRVFKVNTNAYYEMSGLEVSFEELRTFGGHDAKFIDSLQENEFRLYYYNKFKDIASTLNKAKSIVGTTASLQYMKNVFKEKYLLSEDTSGKFSVDKLKFDKLYKMLTEIYTEDNFVKFFKVLNRKTYLNFDKAVFKINIVPKVNYTIYDGFNLRNTNLAANFNGQNTEINNMNFTKLKNFTGLFEF

SEQ ID NO: 10 - protein, 425 aa, Clostridium botulinum
MPFVNKQFNYKDPVNGVDIAYIKIPNAGQMQPVKAFKIHNKIWVIPERDTFTNPEEGDLNPPPEAKQVPVSYYDSTYLSTDNEKDNYLKGVTKLFERIYSTDLGRMLLTSIVRGIPFWGGSTIDTELKVIDTNCINVIQPDGSYRSEELNLVIIGPSADIIQFECKSFGHDVLNLTRNGYGSTQYIRFSPDFTFGFEESLEVDTNPLLGAGKFATDPAVTLAHELIHAEHRLYGIAINPNRVFKVNTNAYYEMSGLEVSFEELRTFGGHDAKFIDSLQENEFRLYYYNKFKDVASTLNKAKSIIGTTASLQYMKNVFKEKYLLSEDTSGKFSVDKLKFDKLYKMLTEIYTEDNFVNFFKVINRKTYLNFDKAVFRINIVPDENYTIKDGFNLKGANLSTNFNGQNTEINSRNFTRLKNFTGLFEF

SEQ ID NO: 11 - protein, 421 aa, Clostridium botulinum
MPFVNKQFNYRDPVNGVDIAYIKIPNAGQMQPVKAFKIHEGVWVIPERDTFTNPEEGDLNPPPEAKQVPVSYYDSTYLSTDNEKDNYLKGVIKLFDRIYSTGLGRMLLSFIVKGIPFWGGSTIDTELKVIDTNCINVIEPGGSYRSEELNLVITGPSADIIQFECKSFGHDVFNLTRNGYGSTQYIRFSPDFTFGFEESLEVDTNPLLGAGTFATDPAVTLAHELIHAAHRLYGIAINPNRVLKVKTNAYYEMSGLEVSFEELRTFGGNDTNFIDSLWQKKFSRDAYDNLQNIARILNEAKTIVGTTTPLQYMKNIFIRKYFLSEDASGKISVNKAAFKEFYRVLTRGFTELEFVNPFKVINRKTYLNFDKAVFRINIVPDENYTINEGFNLEGANSNGQNTEINSRNFTRLKNFTGLFEF

SEQ ID NO: 12 - protein, 425 aa, Clostridium botulinum
MPFVNKQFNYNDPENGVDIAYIKIPNAGKMQPVKAFKIHNKVWVIPERDIFTNPEEVDLNPPPEAKQVPISYYDSAYLSTDNEKDNYLKGVIKLFERIYSTDLGRMLLISIVRGIPFWGGGKIDTELKVIDTNCINIIQLDDSYRSEELNLAIIGPSANIIESQCSSFRDDVLNLTRNGYGSTQYIRFSPDFTVGFEESLEVDTNPLLGAGKFAQDPAVALAHELIHAEHRLYGIAINTNRVFKVNTNAYYEMAGLEVSLEELITFGGNDAKFIDSLQKKEFSLYYYNKFKDIASTLNKAKSIVGTTASLQYMKNVFKEKYLLSEDATGKFLVDRLKFDELYKLLTEIYTEDNFVKFFKVLNRKTYLNFDKAVFKINIVPDVNYTIHDGFNLRNTNLAANFNGQNIEINNKNFDKLKNFTGLFEF

SEQ ID NO: 13 - protein, 425 aa, Clostridium botulinum
MLFVNKQFNYKDPVNGVDIAYIKIPNAGQMQPVKAFKIHNKIWVIPERDTFTNPEEGDLNPPPEAKQVPVSYYDSTYLSTDNEKDNYLKGVTKLFERIYSTELGRMLLTSIVRGIPFWGGSTIDTELKVIDTNCINVIQPDGSYRSEELNLVIIGPSADIIQFECKSFGHDVLNLTRNGYGSTQYIRFSPDFTFGFEESLEVDTNPLLGAGKFATDPAVTLAHELIHAGHRLYGIAINPNRVFKVNTNAYYEMSGLEVSFEELRTFGEHDAKFIDSLQENEFRLYYYNKFKDIASTLNKAKSIVGTTASLQYMKNVFKEKYLLSEDTSGKFSVDKLKFDKLYKMLTEIYTEDNFVKFFKVLNRKTYLNFDKAVFKINIVPEVNYTIYDGFNLRNTNLAANFNGQNTEINNMNFTKLKNFTGLFEF

SEQ ID NO: 14 - protein, 425 aa, Clostridium botulinum
MPFVNKQFNYKDPVNGVDIAYIKIPNAGQMQPVKAFKIHNKIWVIPERDTFTNPEEGDLNPPPEAKQVPVSYYDSTYLSTDNEKDNYLKGVTKLFERIYSTDLGRMLLTSIVRGIPFWGGSTIDTELKVIDTNCINVIQPDGSYRSEELNLVIIGPSADIIQFECKSFGHEVLNLTRNGYGSTQYIRFSPDFTFGFEESLEVDTNPLLGAGKFATDPAVTLAHELIHAGHRLYGIAINPNRVFKVNTNAYYEMSGLEVSFEELRTFGGHDAKFIDSLQENEFRLYYYNKFKDIASTLNKAKSIVGTTASLQYMKNVFKEKYLLSEDTSGKFSVDKLKFDKLYKMLTEIYTEDNFVKFFKVLNRKTYLNFDKAVFKINIVPKVNYTIYDGFNLRNTNLAANFNGQNTEINNMNFAKLKNFTGLFEF

SEQ ID NO: 15 - protein, 425 aa, Clostridium botulinum
MPFVNKQFNYKDPVNGVDIAYIKIPNAGQMQPVKAFKIHNKIWVIPERDIFTNPEEGDLNPPPEAKQVPVSYYDSTYLSTDNEKDNYLKGVTKLFERIYSTDLGRMLLTSIVRGIPFWGGSTIDTELKVIDTNCINVIQPDGSYRSEELNLVIIGPSADIINFECKSFGHDVLNLTRNGYGSTQYIRFSPDFTFGFEESLEVDTNPLLGAGKFAIDPAVTLAHELIHAGHRLYGIAINPNRVFKVNTNAYYEMSGLEVSFEELRTFGGHDAKFIDSLQENEFRLYYYNKFKEVASILNKAKSIIGTTASLQYMKNVFKEKYLLSEDTSGKFSVDKLRFDKLYKMLTEIYTEDNFVKFFKVLNRKTYLNFDKAVFKMNIVPEVNYTIYDGFNLRNTNLAANFNGQNTEINNMNFTKLKNFTGLFEF

SEQ ID NO: 16 - protein, 425 aa, Clostridium botulinum
MPFVNKQFNYKDTVNGIDIAYIKIPNAGQMQPVKAFKIHNKIWVIPERDTFTNPKEGDLNPPPEAKQVPVSYYDSTYLSTDNEKDNYLKGVTKLFERIYSTDLGRMLLTSIVRGIPFWGGSTIDTELKVIDTNCINVIQPDGSYRSEELNLVIIGPSADIIQFECKSFGHDVLNLTRNGYGSTQYIRFSPDFTFGFEESLEVDTNPLLGAGKFATDPAVTLAHELIHAEHRLYGIAINPNRVFKVNTNAYYEMSGLEVSFEELRTFGGHNAKFIDSLQENEFRLYYYNKFKDIASTLNKAKSIVGTTASLQYMKNVFKEKYLLSEDTSGKFSVDKLKFDKLYKMLTEIYTEDNFVKFFKVLNRKTYLNFDKAVFKINIVPDENYTIKDGFNLKNTNLAANFNGQNTEINSRNFTKLKNFTGLFEF

SEQ ID NO: 17 - protein, 871 aa, Clostridium botulinum
YKLLCVRGIITSKTKSLDKGYNKALNDLCIKVNNWDLFFSPSEDNFTNDLNKGEEITSDTNIEAAEENISLDLIQQYYLTFNFDNEPENISIENLSSDIIGQLELMPNIERFPNGKKYELDKYTMFHYLRAQEFEHGKSRIALTNSVNEALLNPSRVYTFFSSDYVKKVNKATEAAMFLGWVEQLVYDFTDETSEVSTTDKIADITIIIPYIGPALNIGNMLYKDDFVGALIFSGAVILLEFIPEIAIPVLGTFALVSYIANKVLTVQTIDNALSKRNEKWDEVYKYIVTNWLAKVNTQIDLIRKKMKEALENQAEATKAIINYQYNQYTEEEKNNINFNIDDLSSKLNESINKAMININKFLNQCSVSYLMNSMIPYGVKRLEDFDASLKDALLKYIYDNRGTLIGQVDRLKDKVNNTLSTDIPFQLSKYVDNQRLLSTFTEYIKNIINTSILNLRYESNHLIDLSRYASKINIGSKVNFDPIDKNQIQLFNLESSKIEVILKNAIVYNSMYENFSTSFWIRIPKYFNSISLNNEYTIINCMENNSGWKVSLNYGEIIWTLQDTQEIKQRVVFKYSQMINISDYINRWIFVTITNNRLNNSKIYINGRLIDQKPISNLGNIHASNNIMFKLDGCRDTHRYIWIKYFNLFDKELNEKEIKDLYDNQSNSGILKDFWGDYLQYDKPYYMLNLYDPNKYVDVNNVGIRGYMYLKGPRGSVMTTNIYLNSSLYRGTKFIIKKYASGNKDNIVRNNDRVYINVVVKNKEYRLATNASQAGVEKILSALEIPDVGNLSQVVVMKSKNDQGITNKCKMNLQDNNGNDIGFIGFHQFNNIAKLVASNWYNRQIERSSRTLGCSWEFIPVDDGWGERPL

SEQ ID NO: 18 - protein, 425 aa, Artificial Sequence
  pBT102
MPFVNKQFNYKDPVNGVDIAYIKIPNAGQMQPVKAFKIHNKIWVIPERDTFTNPEEGDLNPPPEAKQVPVSYYDSTYLSTDNEKDNYLKGVTKLFERIYSTDLGRMLLTSIVRGIPFWGGSTIDTELKVIDTNCINVIQPDGSYRSEELNLVIIGPSADIIQFECKSFGHEVLNLTRNGYGSTQYIRFSPDFTFGFEESLEVDTNPLLGAGKFATDPAVTLAHELIHAGHRLYGIAINPNRVFKVNTNAYYEMSGLEVSFEELRTFGGHDAKFIDSLQENEFRLYYYNKFKDIASTLNKAKSIVGTTASLQYMKNVFKEKYLLSEDTSGKFSVDKLKFDKLYKMLTEIYTEDNFVKFFKVLNRKTYLNFDKAVFKINIVPKVNYTIYDGFNLRNTNLAANFNGQNIEINNKNFDKLKNFTGLFEF

SEQ ID NO: 19 - protein, 425 aa, Artificial Sequence
  pBT103
MPFVNKQFNYKDPVNGVDIAYIKIPNAGQMQPVKAFKIHNKIWVIPERDTFTNPEEGDLNPPPEAKQVPVSYYDSTYLSTDNEKDNYLKGVTKLFERIYSTDLGRMLLTSIVRGIPFWGGSTIDTELKVIDTNCINVIQPDGSYRSEELNLVIIGPSADIIQFECKSFGHEVLNLTRNGYGSTQYIRFSPDFTFGFEESLEVDTNPLLGAGKFATDPAVTLAHELIHAGHRLYGIAINPNRVFKVNTNAYYEMAGLEVSLEELITFGGNDAKFIDSLQKKEFSLYYYNKFKDIASTLNKAKSIVGTTASLQYMKNVFKEKYLLSEDATGKFLVDRLKFDELYKLLTEIYTEDNFVKFFKVLNRKTYLNFDKAVFKINIVPDVNYTIHDGFNLRNTNLAANFNGQNTEINNMNFTKLKNFTGLFEF

SEQ ID NO: 20 - protein, 425 aa, Artificial Sequence
  pBT104
MPFVNKQFNYKDPVNGVDIAYIKIPNAGQMQPVKAFKIHNKIWVIPERDTFTNPEEGDLNPPPEAKQVPVSYYDSTYLSTDNEKDNYLKGVTKLFERIYSTDLGRMLLTSIVRGIPFWGGSTIDTELKVIDTNCINVIQPDGSYRSEELNLVIIGPSADIIQFECKSFGHEVLNLTRNGYGSTQYIRFSPDFTFGFEESLEVDTNPLLGAGKFATDPAVTLAHELIHAGHRLYGIAINPNRVFKVNTNAYYEMAGLEVSLEELITFGGNDAKFIDSLQKKEFSLYYYNKFKDIASTLNKAKSIVGTTASLQYMKNVFKEKYLLSEDATGKFLVDRLKFDELYKLLTEIYTEDNFVKFFKVLNRKTYLNFDKAVFKINIVPDVNYTIHDGFNLRNTNLAANFNGQNIEINNKNFDKLKNFTGLFEF

SEQ ID NO: 21 - protein, 425 aa, Artificial Sequence
  pBT105
MPFVNKQFNYKDPVNGVDIAYIKIPNAGQMQPVKAFKIHNKIWVIPERDTFTNPEEGDLNPPPEAKQVPVSYYDSTYLSTDNEKDNYLKGVTKLFERIYSTDLGRMLLTSIVRGIPFWGGGKIDTELKVIDTNCINIIQLDDSYRSEELNLAIIGPSANIIESQCSSFRDDVLNLTRNGYGSTQYIRFSPDFTVGFEESLEVDTNPLLGAGKFAQDPAVALAHELIHAEHRLYGIAINTNRVFKVNTNAYYEMAGLEVSLEELITFGGNDAKFIDSLQKKEFSLYYYNKFKDIASTLNKAKSIVGTTASLQYMKNVFKEKYLLSEDATGKFLVDRLKFDELYKLLTEIYTEDNFVKFFKVLNRKTYLNFDKAVFKINIVPDVNYTIHDGFNLRNTNLAANFNGQNIEINNKNFDKLKNFTGLFEF

SEQ ID NO: 22 - protein, 425 aa, Artificial Sequence
  pBT106
MPFVNKQFNYKDPVNGVDIAYIKIPNAGQMQPVKAFKIHNKIWVIPERDTFTNPEEGDLNPPPEAKQVPVSYYDSTYLSTDNEKDNYLKGVTKLFERIYSTDLGRMLLTSIVRGIPFWGGGKIDTELKVIDTNCINIIQLDDSYRSEELNLAIIGPSANIIESQCSSFRDDVLNLTRNGYGSTQYIRFSPDFTVGFEESLEVDTNPLLGAGKFAQDPAVALAHELIHAEHRLYGIAINTNRVFKVNTNAYYEMAGLEVSLEELITFGGNDAKFIDSLQKKEFSLYYYNKFKDIASTLNKAKSIVGTTASLQYMKNVFKEKYLLSEDATGKFLVDRLKFDELYKLLTEIYTEDNFVKFFKVLNRKTYLNFDKAVFKINIVPDVNYTIHDGFNLRNTNLAANFNGQNTEINNMNFTKLKNFTGLFEF

SEQ ID NO: 23 - protein, 425 aa, Artificial Sequence
  pBT107
MPFVNKQFNYKDPVNGVDIAYIKIPNAGQMQPVKAFKIHNKIWVIPERDTFTNPEEGDLNPPPEAKQVPVSYYDSTYLSTDNEKDNYLKGVTKLFERIYSTDLGRMLLTSIVRGIPFWGGGKIDTELKVIDTNCINIIQLDDSYRSEELNLAIIGPSANIIESQCSSFRDDVLNLTRNGYGSTQYIRFSPDFTVGFEESLEVDTNPLLGAGKFAQDPAVALAHELIHAEHRLYGIAINTNRVFKVNTNAYYEMSGLEVSFEELRTFGGHDAKFIDSLQENEFRLYYYNKFKDIASTLNKAKSIVGTTASLQYMKNVFKEKYLLSEDTSGKFSVDKLKFDKLYKMLTEIYTEDNFVKFFKVLNRKTYLNFDKAVFKINIVPKVNYTIYDGFNLRNTNLAANFNGQNTEINNMNFTKLKNFTGLFEF

SEQ ID NO: 24 - protein, 425 aa, Artificial Sequence
  pBT108
MPFVNKQFNYKDPVNGVDIAYIKIPNAGQMQPVKAFKIHNKIWVIPERDTFTNPEEGDLNPPPEAKQVPVSYYDSTYLSTDNEKDNYLKGVTKLFERIYSTDLGRMLLTSIVRGIPFWGGGKIDTELKVIDTNCINIIQLDDSYRSEELNLAIIGPSANIIESQCSSFRDDVLNLTRNGYGSTQYIRFSPDFTVGFEESLEVDTNPLLGAGKFAQDPAVALAHELIHAEHRLYGIAINTNRVFKVNTNAYYEMSGLEVSFEELRTFGGHDAKFIDSLQENEFRLYYYNKFKDIASTLNKAKSIVGTTASLQYMKNVFKEKYLLSEDTSGKFSVDKLKFDKLYKMLTEIYTEDNFVKFFKVLNRKTYLNFDKAVFKINIVPKVNYTIYDGFNLRNTNLAANFNGQNIEINNKNFDKLKNFTGLFEF

SEQ ID NO: 25 - protein, 425 aa, Artificial Sequence
  pBT109
MPFVNKQFNYNDPENGVDIAYIKIPNAGKMQPVKAFKIHNKVWVIPERDIFTNPEEVDLNPPPEAKQVPISYYDSAYLSTDNEKDNYLKGVIKLFERIYSTDLGRMLLISIVRGIPFWGGGKIDTELKVIDTNCINIIQLDDSYRSEELNLAIIGPSANIIESQCSSFRDDVLNLTRNGYGSTQYIRFSPDFTVGFEESLEVDTNPLLGAGKFAQDPAVALAHELIHAEHRLYGIAINTNRVFKVNTNAYYEMAGLEVSLEELITFGGNDAKFIDSLQKKEFSLYYYNKFKDIASTLNKAKSIVGTTASLQYMKNVFKEKYLLSEDATGKFLVDRLKFDELYKLLTEIYTEDNFVKFFKVLNRKTYLNFDKAVFKINIVPDVNYTIHDGFNLRNTNLAANFNGQNTEINNMNFTKLKNFTGLFEF

SEQ ID NO: 26 - protein, 425 aa, Artificial Sequence
  pBT110
MPFVNKQFNYNDPENGVDIAYIKIPNAGKMQPVKAFKIHNKVWVIPERDIFTNPEEVDLNPPPEAKQVPISYYDSAYLSTDNEKDNYLKGVIKLFERIYSTDLGRMLLISIVRGIPFWGGGKIDTELKVIDTNCINIIQLDDSYRSEELNLAIIGPSANIIESQCSSFRDDVLNLTRNGYGSTQYIRFSPDFTVGFEESLEVDTNPLLGAGKFAQDPAVALAHELIHAEHRLYGIAINTNRVFKVNTNAYYEMSGLEVSFEELRTFGGHDAKFIDSLQENEFRLYYYNKFKDIASTLNKAKSIVGTTASLQYMKNVFKEKYLLSEDTSGKFSVDKLKFDKLYKMLTEIYTEDNFVKFFKVLNRKTYLNFDKAVFKINIVPKVNYTIYDGFNLRNTNLAANFNGQNTEINNMNFTKLKNFTGLFEF

SEQ ID NO: 27 - protein, 425 aa, Artificial Sequence
  pBT111
MPFVNKQFNYNDPENGVDIAYIKIPNAGKMQPVKAFKIHNKVWVIPERDIFTNPEEVDLNPPPEAKQVPISYYDSAYLSTDNEKDNYLKGVIKLFERIYSTDLGRMLLISIVRGIPFWGGGKIDTELKVIDTNCINIIQLDDSYRSEELNLAIIGPSANIIESQCSSFRDDVLNLTRNGYGSTQYIRFSPDFTVGFEESLEVDTNPLLGAGKFAQDPAVALAHELIHAEHRLYGIAINTNRVFKVNTNAYYEMSGLEVSFEELRTFGGHDAKFIDSLQENEFRLYYYNKFKDIASTLNKAKSIVGTTASLQYMKNVFKEKYLLSEDTSGKFSVDKLKFDKLYKMLTEIYTEDNFVKFFKVLNRKTYLNFDKAVFKINIVPKVNYTIYDGFNLRNTNLAANFNGQNIEINNKNFDKLKNFTGLFEF

SEQ ID NO: 28 - protein, 425 aa, Artificial Sequence
  pBT112
MPFVNKQFNYNDPENGVDIAYIKIPNAGKMQPVKAFKIHNKVWVIPERDIFTNPEEVDLNPPPEAKQVPISYYDSAYLSTDNEKDNYLKGVIKLFERIYSTDLGRMLLISIVRGIPFWGGSTIDTELKVIDTNCINVIQPDGSYRSEELNLVIIGPSADIIQFECKSFGHEVLNLTRNGYGSTQYIRFSPDFTFGFEESLEVDTNPLLGAGKFATDPAVTLAHELIHAGHRLYGIAINPNRVFKVNTNAYYEMSGLEVSFEELRTFGGHDAKFIDSLQENEFRLYYYNKFKDIASTLNKAKSIVGTTASLQYMKNVFKEKYLLSEDTSGKFSVDKLKFDKLYKMLTEIYTEDNFVKFFKVLNRKTYLNFDKAVFKINIVPKVNYTIYDGFNLRNTNLAANFNGQNIEINNKNFDKLKNFTGLFEF

SEQ ID NO: 29 - protein, 425 aa, Artificial Sequence
  pBT113
MPFVNKQFNYNDPENGVDIAYIKIPNAGKMQPVKAFKIHNKVWVIPERDIFTNPEEVDLNPPPEAKQVPISYYDSAYLSTDNEKDNYLKGVIKLFERIYSTDLGRMLLISIVRGIPFWGGSTIDTELKVIDTNCINVIQPDGSYRSEELNLVIIGPSADIIQFECKSFGHEVLNLTRNGYGSTQYIRFSPDFTFGFEESLEVDTNPLLGAGKFATDPAVTLAHELIHAGHRLYGIAINPNRVFKVNTNAYYEMSGLEVSFEELRTFGGHDAKFIDSLQENEFRLYYYNKFKDIASTLNKAKSIVGTTASLQYMKNVFKEKYLLSEDTSGKFSVDKLKFDKLYKMLTEIYTEDNFVKFFKVLNRKTYLNFDKAVFKINIVPKVNYTIYDGFNLRNTNLAANFNGQNTEINNMNFTKLKNFTGLFEF

SEQ ID NO: 30 - protein, 425 aa, Artificial Sequence
  pBT114
MPFVNKQFNYNDPENGVDIAYIKIPNAGKMQPVKAFKIHNKVWVIPERDIFTNPEEVDLNPPPEAKQVPISYYDSAYLSTDNEKDNYLKGVIKLFERIYSTDLGRMLLISIVRGIPFWGGSTIDTELKVIDTNCINVIQPDGSYRSEELNLVIIGPSADIIQFECKSFGHEVLNLTRNGYGSTQYIRFSPDFTFGFEESLEVDTNPLLGAGKFATDPAVTLAHELIHAGHRLYGIAINPNRVFKVNTNAYYEMAGLEVSLEELITFGGNDAKFIDSLQKKEFSLYYYNKFKDIASTLNKAKSIVGTTASLQYMKNVFKEKYLLSEDATGKFLVDRLKFDELYKLLTEIYTEDNFVKFFKVLNRKTYLNFDKAVFKINIVPDVNYTIHDGFNLRNTNLAANFNGQNIEINNKNFDKLKNFTGLFEF

SEQ ID NO: 31 - protein, 425 aa, Artificial Sequence
  pBT115
MPFVNKQFNYNDPENGVDIAYIKIPNAGKMQPVKAFKIHNKVWVIPERDIFTNPEEVDLNPPPEAKQVPISYYDSAYLSTDNEKDNYLKGVIKLFERIYSTDLGRMLLISIVRGIPFWGGSTIDTELKVIDTNCINVIQPDGSYRSEELNLVIIGPSADIIQFECKSFGHEVLNLTRNGYGSTQYIRFSPDFTFGFEESLEVDTNPLLGAGKFATDPAVTLAHELIHAGHRLYGIAINPNRVFKVNTNAYYEMAGLEVSLEELITFGGNDAKFIDSLQKKEFSLYYYNKFKDIASTLNKAKSIVGTTASLQYMKNVFKEKYLLSEDATGKFLVDRLKFDELYKLLTEIYTEDNFVKFFKVLNRKTYLNFDKAVFKINIVPDVNYTIHDGFNLRNTNLAANFNGQNTEINNMNFTKLKNFTGLFEF

SEQ ID NO: 32 - protein, 425 aa, Artificial Sequence
  pBT158
MPFVNKQFNYKDPVNGVDIAYIKIPNAGQMQPVKAFKIHNKIWVIPERDTFTNPEEGDLNPPPEAKQVPVSYYDSTYLSTDNEKDNYLKGVTKLFERIYSTDLGRMLLTSIVRGIPFWGGSTIDTELKVIDTNCINVIQPDGSYRSEELNLVIIGPSADIIQFECKSFGHEVLNLTRNGYGSTQYIRFSPDFTFGFEESLEVDTNPLLGAGKFATDPAVTLAHELIHAGHRLYGIAINPNRVFKVNTNAYYEMSGLEVSFEELRTFGGHDAKFIDSLQENEFRLYYYNKFKDVASTLNKAKSIIGTTASLQYMKNVFKEKYLLSEDTSGKFSVDKLKFDKLYKMLTEIYTEDNFVNFFKVINRKTYLNFDKAVFRINIVPDENYTIKDGFNLKGANLAANFNGQNTEINNMNFTKLKNFTGLFEF

SEQ ID NO: 33 - protein, 425 aa, Artificial Sequence
  pBT160
MPFVNKQFNYKDPVNGVDIAYIKIPNAGQMQPVKAFKIHNKIWVIPERDTFTNPEEGDLNPPPEAKQVPVSYYDSTYLSTDNEKDNYLKGVTKLFERIYSTDLGRMLLTSIVRGIPFWGGSTIDTELKVIDTNCINVIQPDGSYRSEELNLVIIGPSADIIQFECKSFGHEVLNLTRNGYGSTQYIRFSPDFTFGFEESLEVDTNPLLGAGKFATDPAVTLAHELIHAGHRLYGIAINPNRVFKVNTNAYYEMSGLEVSFEELRTFGEHDAKFIDSLQENEFRLYYYNKFKDIASTLNKAKSIVGTTASLQYMKNVFKEKYLLSEDTSGKFSVDKLKFDKLYKMLTEIYTEDNFVKFFKVLNRKTYLNFDKAVFKINIVPEVNYTIYDGFNLRNTNLAANFNGQNTEINNMNFTKLKNFTGLFEF

SEQ ID NO: 34 - protein, 425 aa, Artificial Sequence
  pBT161
MPFVNKQFNYKDPVNGVDIAYIKIPNAGQMQPVKAFKIHNKIWVIPERDTFTNPEEGDLNPPPEAKQVPVSYYDSTYLSTDNEKDNYLKGVTKLFERIYSTDLGRMLLTSIVRGIPFWGGSTIDTELKVIDTNCINVIQPDGSYRSEELNLVIIGPSADIIQFECKSFGHEVLNLTRNGYGSTQYIRFSPDFTFGFEESLEVDTNPLLGAGKFATDPAVTLAHELIHAGHRLYGIAINPNRVFKVNTNAYYEMSGLEVSFEELRTFGGHDAKFIDSLQENEFRLYYYNKFKEVASILNKAKSIIGTTASLQYMKNVFKEKYLLSEDTSGKFSVDKLRFDKLYKMLTEIYTEDNFVKFFKVLNRKTYLNFDKAVFKMNIVPEVNYTIYDGFNLRNTNLAANFNGQNTEINNMNFTKLKNFTGLFEF

SEQ ID NO: 35 - protein, 425 aa, Artificial Sequence
  pBT162
MPFVNKQFNYKDPVNGVDIAYIKIPNAGQMQPVKAFKIHNKIWVIPERDTFTNPEEGDLNPPPEAKQVPVSYYDSTYLSTDNEKDNYLKGVTKLFERIYSTDLGRMLLTSIVRGIPFWGGSTIDTELKVIDTNCINVIQPDGSYRSEELNLVIIGPSADIIQFECKSFGHEVLNLTRNGYGSTQYIRFSPDFTFGFEESLEVDTNPLLGAGKFATDPAVTLAHELIHAGHRLYGIAINPNRVFKVNTNAYYEMSGLEVSFEELRTFGGHNAKFIDSLQENEFRLYYYNKFKDIASTLNKAKSIVGTTASLQYMKNVFKEKYLLSEDTSGKFSVDKLKFDKLYKMLTEIYTEDNFVKFFKVLNRKTYLNFDKAVFKINIVPDENYTIKDGFNLKNTNLAANFNGQNTEINNMNFTKLKNFTGLFEF

SEQ ID NO: 36 - protein, 1296 aa, Artificial Sequence
  pBT142
MPFVNKQFNYKDPVNGVDIAYIKIPNAGQMQPVKAFKIHNKIWVIPERDTFTNPEEGDLNPPPEAKQVPVSYYDSTYLSTDNEKDNYLKGVTKLFERIYSTDLGRMLLTSIVRGIPFWGGSTIDTELKVIDTNCINVIQPDGSYRSEELNLVIIGPSADIIQFECKSFGHEVLNLTRNGYGSTQYIRFSPDFTFGFEESLEVDTNPLLGAGKFATDPAVTLAHELIHAGHRLYGIAINPNRVFKVNTNAYYEMAGLEVSLEELITFGGNDAKFIDSLQKKEFSLYYYNKFKDIASTLNKAKSIVGTTASLQYMKNVFKEKYLLSEDATGKFLVDRLKFDELYKLLTEIYTEDNFVKFFKVLNRKTYLNFDKAVFKINIVPDVNYTIHDGFNLRNTNLAANFNGQNTEINNMNFTKLKNFTGLFEFYKLLCVRGIITSKTKSLDKGYNKALNDLCIKVNNWDLFFSPSEDNFTNDLNKGEEITSDTNIEAAEENISLDLIQQYYLTFNFDNEPENISIENLSSDIIGQLELMPNIERFPNGKKYELDKYTMFHYLRAQEFEHGKSRIALTNSVNEALLNPSRVYTFFSSDYVKKVNKATEAAMFLGWVEQLVYDFTDETSEVSTTDKIADITIIIPYIGPALNIGNMLYKDDFVGALIFSGAVILLEFIPEIAIPVLGTFALVSYIANKVLTVQTIDNALSKRNEKWDEVYKYIVTNWLAKVNTQIDLIRKKMKEALENQAEATKAIINYQYNQYTEEEKNNINFNIDDLSSKLNESINKAMININKFLNQCSVSYLMNSMIPYGVKRLEDFDASLKDALLKYIYDNRGTLIGQVDRLKDKVNNTLSTDIPFQLSKYVDNQRLLSTFTEYIKNIINTSILNLRYESNHLIDLSRYASKINIGSKVNFDPIDKNQIQLFNLESSKIEVILKNAIVYNSMYENFSTSFWIRIPKYFNSISLNNEYTIINCMENNSGWKVSLNYGEIIWTLQDTQEIKQRVVFKYSQMINISDYINRWIFVTITNNRLNNSKIYINGRLIDQKPISNLGNIHASNNIMFKLDGCRDTHRYIWIKYFNLFDKELNEKEIKDLYDNQSNSGILKDFWGDYLQYDKPYYMLNLYDPNKYVDVNNVGIRGYMYLKGPRGSVMTTNIYLNSSLYRGTKFIIKKYASGNKDNIVRNNDRVYINVVVKNKEYRLATNASQAGVEKILSALEIPDVGNLSQVVVMKSKNDQGITNKCKMNLQDNNGNDIGFIGFHQFNNIAKLVASNWYNRQIERSSRTLGCSWEFIPVDDGWGERPL

SEQ ID NO: 37 - protein, 1296 aa, Artificial Sequence
  pBT143
MPFVNKQFNYNDPENGVDIAYIKIPNAGKMQPVKAFKIHNKVWVIPERDIFTNPEEVDLNPPPEAKQVPISYYDSAYLSTDNEKDNYLKGVIKLFERIYSTDLGRMLLISIVRGIPFWGGSTIDTELKVIDTNCINVIQPDGSYRSEELNLVIIGPSADIIQFECKSFGHEVLNLTRNGYGSTQYIRFSPDFTFGFEESLEVDTNPLLGAGKFATDPAVTLAHELIHAGHRLYGIAINPNRVFKVNTNAYYEMSGLEVSFEELRTFGGHDAKFIDSLQENEFRLYYYNKFKDIASTLNKAKSIVGTTASLQYMKNVFKEKYLLSEDTSGKFSVDKLKFDKLYKMLTEIYTEDNFVKFFKVLNRKTYLNFDKAVFKINIVPKVNYTIYDGFNLRNTNLAANFNGQNIEINNKNFDKLKNFTGLFEFYKLLCVRGIITSKTKSLDKGYNKALNDLCIKVNNWDLFFSPSEDNFTNDLNKGEEITSDTNIEAAEENISLDLIQQYYLTFNFDNEPENISIENLSSDIIGQLELMPNIERFPNGKKYELDKYTMFHYLRAQEFEHGKSRIALTNSVNEALLNPSRVYTFFSSDYVKKVNKATEAAMFLGWVEQLVYDFTDETSEVSTTDKIADITIIIPYIGPALNIGNMLYKDDFVGALIFSGAVILLEFIPEIAIPVLGTFALVSYIANKVLTVQTIDNALSKRNEKWDEVYKYIVTNWLAKVNTQIDLIRKKMKEALENQAEATKAIINYQYNQYTEEEKNNINFNIDDLSSKLNESINKAMININKFLNQCSVSYLMNSMIPYGVKRLEDFDASLKDALLKYIYDNRGTLIGQVDRLKDKVNNTLSTDIPFQLSKYVDNQRLLSTFTEYIKNIINTSILNLRYESNHLIDLSRYASKINIGSKVNFDPIDKNQIQLFNLESSKIEVILKNAIVYNSMYENFSTSFWIRIPKYFNSISLNNEYTIINCMENNSGWKVSLNYGEIIWTLQDTQEIKQRVVFKYSQMINISDYINRWIFVTITNNRLNNSKIYINGRLIDQKPISNLGNIHASNNIMFKLDGCRDTHRYIWIKYFNLFDKELNEKEIKDLYDNQSNSGILKDFWGDYLQYDKPYYMLNLYDPNKYVDVNNVGIRGYMYLKGPRGSVMTTNIYLNSSLYRGTKFIIKKYASGNKDNIVRNNDRVYINVVVKNKEYRLATNASQAGVEKILSALEIPDVGNLSQVVVMKSKNDQGITNKCKMNLQDNNGNDIGFIGFHQFNNIAKLVASNWYNRQIERSSRTLGCSWEFIPVDDGWGERPL

SEQ ID NO: 38 - protein, 1296 aa, Artificial Sequence
  pBT144
MPFVNKQFNYNDPENGVDIAYIKIPNAGKMQPVKAFKIHNKVWVIPERDIFTNPEEVDLNPPPEAKQVPISYYDSAYLSTDNEKDNYLKGVIKLFERIYSTDLGRMLLISIVRGIPFWGGSTIDTELKVIDTNCINVIQPDGSYRSEELNLVIIGPSADIIQFECKSFGHEVLNLTRNGYGSTQYIRFSPDFTFGFEESLEVDTNPLLGAGKFATDPAVTLAHELIHAGHRLYGIAINPNRVFKVNTNAYYEMSGLEVSFEELRTFGGHDAKFIDSLQENEFRLYYYNKFKDIASTLNKAKSIVGTTASLQYMKNVFKEKYLLSEDTSGKFSVDKLKFDKLYKMLTEIYTEDNFVKFFKVLNRKTYLNFDKAVFKINIVPKVNYTIYDGFNLRNTNLAANFNGQNTEINNMNFTKLKNFTGLFEFYKLLCVRGIITSKTKSLDKGYNKALNDLCIKVNNWDLFFSPSEDNFTNDLNKGEEITSDTNIEAAEENISLDLIQQYYLTFNFDNEPENISIENLSSDIIGQLELMPNIERFPNGKKYELDKYTMFHYLRAQEFEHGKSRIALTNSVNEALLNPSRVYTFFSSDYVKKVNKATEAAMFLGWVEQLVYDFTDETSEVSTTDKIADITIIIPYIGPALNIGNMLYKDDFVGALIFSGAVILLEFIPEIAIPVLGTFALVSYIANKVLTVQTIDNALSKRNEKWDEVYKYIVTNWLAKVNTQIDLIRKKMKEALENQAEATKAIINYQYNQYTEEEKNNINFNIDDLSSKLNESINKAMININKFLNQCSVSYLMNSMIPYGVKRLEDFDASLKDALLKYIYDNRGTLIGQVDRLKDKVNNTLSTDIPFQLSKYVDNQRLLSTFTEYIKNIINTSILNLRYESNHLIDLSRYASKINIGSKVNFDPIDKNQIQLFNLESSKIEVILKNAIVYNSMYENFSTSFWIRIPKYFNSISLNNEYTIINCMENNSGWKVSLNYGEIIWTLQDTQEIKQRVVFKYSQMINISDYINRWIFVTITNNRLNNSKIYINGRLIDQKPISNLGNIHASNNIMFKLDGCRDTHRYIWIKYFNLFDKELNEKEIKDLYDNQSNSGILKDFWGDYLQYDKPYYMLNLYDPNKYVDVNNVGIRGYMYLKGPRGSVMTTNIYLNSSLYRGTKFIIKKYASGNKDNIVRNNDRVYINVVVKNKEYRLATNASQAGVEKILSALEIPDVGNLSQVVVMKSKNDQGITNKCKMNLQDNNGNDIGFIGFHQFNNIAKLVASNWYNRQIERSSRTLGCSWEFIPVDDGWGERPL

SEQ ID NO: 39 - protein, 1296 aa, Artificial Sequence
  pBT145
MPFVNKQFNYNDPENGVDIAYIKIPNAGKMQPVKAFKIHNKVWVIPERDIFTNPEEVDLNPPPEAKQVPISYYDSAYLSTDNEKDNYLKGVIKLFERIYSTDLGRMLLISIVRGIPFWGGSTIDTELKVIDTNCINVIQPDGSYRSEELNLVIIGPSADIIQFECKSFGHEVLNLTRNGYGSTQYIRFSPDFTFGFEESLEVDTNPLLGAGKFATDPAVTLAHELIHAGHRLYGIAINPNRVFKVNTNAYYEMAGLEVSLEELITFGGNDAKFIDSLQKKEFSLYYYNKFKDIASTLNKAKSIVGTTASLQYMKNVFKEKYLLSEDATGKFLVDRLKFDELYKLLTEIYTEDNFVKFFKVLNRKTYLNFDKAVFKINIVPDVNYTIHDGFNLRNTNLAANFNGQNIEINNKNFDKLKNFTGLFEFYKLLCVRGIITSKTKSLDKGYNKALNDLCIKVNNWDLFFSPSEDNFTNDLNKGEEITSDTNIEAAEENISLDLIQQYYLTFNFDNEPENISIENLSSDIIGQLELMPNIERFPNGKKYELDKYTMFHYLRAQEFEHGKSRIALTNSVNEALLNPSRVYTFFSSDYVKKVNKATEAAMFLGWVEQLVYDFTDETSEVSTTDKIADITIIIPYIGPALNIGNMLYKDDFVGALIFSGAVILLEFIPEIAIPVLGTFALVSYIANKVLTVQTIDNALSKRNEKWDEVYKYIVTNWLAKVNTQIDLIRKKMKEALENQAEATKAIINYQYNQYTEEEKNNINFNIDDLSSKLNESINKAMININKFLNQCSVSYLMNSMIPYGVKRLEDFDASLKDALLKYIYDNRGTLIGQVDRLKDKVNNTLSTDIPFQLSKYVDNQRLLSTFTEYIKNIINTSILNLRYESNHLIDLSRYASKINIGSKVNFDPIDKNQIQLFNLESSKIEVILKNAIVYNSMYENFSTSFWIRIPKYFNSISLNNEYTIINCMENNSGWKVSLNYGEIIWTLQDTQEIKQRVVFKYSQMINISDYINRWIFVTITNNRLNNSKIYINGRLIDQKPISNLGNIHASNNIMFKLDGCRDTHRYIWIKYFNLFDKELNEKEIKDLYDNQSNSGILKDFWGDYLQYDKPYYMLNLYDPNKYVDVNNVGIRGYMYLKGPRGSVMTTNIYLNSSLYRGTKFIIKKYASGNKDNIVRNNDRVYINVVVKNKEYRLATNASQAGVEKILSALEIPDVGNLSQVVVMKSKNDQGITNKCKMNLQDNNGNDIGFIGFHQFNNIAKLVASNWYNRQIERSSRTLGCSWEFIPVDDGWGERPL

SEQ ID NO: 40 - protein, 1296 aa, Artificial Sequence
  pBT146
MPFVNKQFNYNDPENGVDIAYIKIPNAGKMQPVKAFKIHNKVWVIPERDIFTNPEEVDLNPPPEAKQVPISYYDSAYLSTDNEKDNYLKGVIKLFERIYSTDLGRMLLISIVRGIPFWGGSTIDTELKVIDTNCINVIQPDGSYRSEELNLVIIGPSADIIQFECKSFGHEVLNLTRNGYGSTQYIRFSPDFTFGFEESLEVDTNPLLGAGKFATDPAVTLAHELIHAGHRLYGIAINPNRVFKVNTNAYYEMAGLEVSLEELITFGGNDAKFIDSLQKKEFSLYYYNKFKDIASTLNKAKSIVGTTASLQYMKNVFKEKYLLSEDATGKFLVDRLKFDELYKLLTEIYTEDNFVKFFKVLNRKTYLNFDKAVFKINIVPDVNYTIHDGFNLRNTNLAANFNGQNTEINNMNFTKLKNFTGLFEFYKLLCVRGIITSKTKSLDKGYNKALNDLCIKVNNWDLFFSPSEDNFTNDLNKGEEITSDTNIEAAEENISLDLIQQYYLTFNFDNEPENISIENLSSDIIGQLELMPNIERFPNGKKYELDKYTMFHYLRAQEFEHGKSRIALTNSVNEALLNPSRVYTFFSSDYVKKVNKATEAAMFLGWVEQLVYDFTDETSEVSTTDKIADITIIIPYIGPALNIGNMLYKDDFVGALIFSGAVILLEFIPEIAIPVLGTFALVSYIANKVLTVQTIDNALSKRNEKWDEVYKYIVTNWLAKVNTQIDLIRKKMKEALENQAEATKAIINYQYNQYTEEEKNNINFNIDDLSSKLNESINKAMININKFLNQCSVSYLMNSMIPYGVKRLEDFDASLKDALLKYIYDNRGTLIGQVDRLKDKVNNTLSTDIPFQLSKYVDNQRLLSTFTEYIKNIINTSILNLRYESNHLIDLSRYASKINIGSKVNFDPIDKNQIQLFNLESSKIEVILKNAIVYNSMYENFSTSFWIRIPKYFNSISLNNEYTIINCMENNSGWKVSLNYGEIIWTLQDTQEIKQRVVFKYSQMINISDYINRWIFVTITNNRLNNSKIYINGRLIDQKPISNLGNIHASNNIMFKLDGCRDTHRYIWIKYFNLFDKELNEKEIKDLYDNQSNSGILKDFWGDYLQYDKPYYMLNLYDPNKYVDVNNVGIRGYMYLKGPRGSVMTTNIYLNSSLYRGTKFIIKKYASGNKDNIVRNNDRVYINVVVKNKEYRLATNASQAGVEKILSALEIPDVGNLSQVVVMKSKNDQGITNKCKMNLQDNNGNDIGFIGFHQFNNIAKLVASNWYNRQIERSSRTLGCSWEFIPVDDGWGERPL

SEQ ID NO: 41 - protein, 1296 aa, Artificial Sequence
  pBT147
MPFVNKQFNYKDPVNGVDIAYIKIPNAGQMQPVKAFKIHNKIWVIPERDTFTNPEEGDLNPPPEAKQVPVSYYDSTYLSTDNEKDNYLKGVTKLFERIYSTDLGRMLLTSIVRGIPFWGGSTIDTELKVIDTNCINVIQPDGSYRSEELNLVIIGPSADIIQFECKSFGHEVLNLTRNGYGSTQYIRFSPDFTFGFEESLEVDTNPLLGAGKFATDPAVTLAHELIHAGHRLYGIAINPNRVFKVNTNAYYEMAGLEVSLEELITFGGNDAKFIDSLQKKEFSLYYYNKFKDIASTLNKAKSIVGTTASLQYMKNVFKEKYLLSEDATGKFLVDRLKFDELYKLLTEIYTEDNFVKFFKVLNRKTYLNFDKAVFKINIVPDVNYTIHDGFNLRNTNLAANFNGQNIEINNKNFDKLKNFTGLFEFYKLLCVRGIITSKTKSLDKGYNKALNDLCIKVNNWDLFFSPSEDNFTNDLNKGEEITSDTNIEAAEENISLDLIQQYYLTFNFDNEPENISIENLSSDIIGQLELMPNIERFPNGKKYELDKYTMFHYLRAQEFEHGKSRIALTNSVNEALLNPSRVYTFFSSDYVKKVNKATEAAMFLGWVEQLVYDFTDETSEVSTTDKIADITIIIPYIGPALNIGNMLYKDDFVGALIFSGAVILLEFIPEIAIPVLGTFALVSYIANKVLTVQTIDNALSKRNEKWDEVYKYIVTNWLAKVNTQIDLIRKKMKEALENQAEATKAIINYQYNQYTEEEKNNINFNIDDLSSKLNESINKAMININKFLNQCSVSYLMNSMIPYGVKRLEDFDASLKDALLKYIYDNRGTLIGQVDRLKDKVNNTLSTDIPFQLSKYVDNQRLLSTFTEYIKNIINTSILNLRYESNHLIDLSRYASKINIGSKVNFDPIDKNQIQLFNLESSKIEVILKNAIVYNSMYENFSTSFWIRIPKYFNSISLNNEYTIINCMENNSGWKVSLNYGEIIWTLQDTQEIKQRVVFKYSQMINISDYINRWIFVTITNNRLNNSKIYINGRLIDQKPISNLGNIHASNNIMFKLDGCRDTHRYIWIKYFNLFDKELNEKEIKDLYDNQSNSGILKDFWGDYLQYDKPYYMLNLYDPNKYVDVNNVGIRGYMYLKGPRGSVMTTNIYLNSSLYRGTKFIIKKYASGNKDNIVRNNDRVYINVVVKNKEYRLATNASQAGVEKILSALEIPDVGNLSQVVVMKSKNDQGITNKCKMNLQDNNGNDIGFIGFHQFNNIAKLVASNWYNRQIERSSRTLGCSWEFIPVDDGWGERPL